European Patent Application EP 4 471 136 A1, published December 4, 2024. Title: D-AMINO ACID OXIDASE AND USE THEREOF IN PREPARATION OF L-PHOSPHINOTHRICIN OR INTERMEDIATE THEREOF. Applicant: SHANGHAI QIZHOU ZIYUE BIOTECHNOLOGY CO., LTD. Application CN PCT/CN/2023/073897, filed January 30, 2023. The sequence listing filed with the application follows.

SEQUENCE LISTING (12 sequences)

SEQ ID NO: 1 - protein, 372 aa, synthetic construct
MTQNKRVVVLGSGVIGLSCALALAQKGYKVHVVARDLPEDTVAQTFASPWAGAAWNPHMSKEAGPRQAKWEEATFKQWVDFVPQGLAMWLKGTRRFAETEADLLGHWYKDIVPNYRHLNPSDCPPGAIGVTYDTLSVNAPKFCQYLQREAQKLGVTFERRLVTSLEQIADGADLIVNATGLGAKSIAGVEDQEVEPIRGQTVLIKSNCKRLTTDSSDPKSPAYIIPRPGGEVICGGTYLVGNYDLSVDPATIPRILKHCLRLDPSISTDGTLEGIEILRHNVGLRPARRGGPRVELERVSFPLKRGQSLLALGTAKAAEGKASRTVPVVHAYGFSSAGYQQGWGAALEVRDLVDQAIGSSSSASSGRYLAKL

SEQ ID NO: 2 - DNA, 41 bp, synthetic construct
  misc_feature 21..22: note = n is a, c, g, or t
  source 1..41: mol_type = other DNA
ctttagcccagaagggctatnnkgtgcatgtggttgcccgc

SEQ ID NO: 3 - DNA, 41 bp, synthetic construct
  misc_feature 20..21: note = n is a, c, g, or t
  source 1..41: mol_type = other DNA
gcgggcaaccacatgcacmnnatagcccttctgggctaaag

SEQ ID NO: 4 - DNA, 39 bp, synthetic construct
  misc_feature 19..20: note = n is a, c, g, or t
  source 1..39: mol_type = other DNA
gatctgccggaagacacannkgcccagacctttgcaagc

SEQ ID NO: 5 - DNA, 39 bp, synthetic construct
  misc_feature 20..21: note = n is a, c, g, or t
  source 1..39: mol_type = other DNA
gcttgcaaaggtctgggcmnntgtgtcttccggcagatc

SEQ ID NO: 6 - DNA, 40 bp, synthetic construct
  misc_feature 19..20: note = n is a, c, g, or t
  source 1..40: mol_type = other DNA
gtggaagatcaagaagtgnnkcctatccgcggccaaacag

SEQ ID NO: 7 - DNA, 40 bp, synthetic construct
  misc_feature 21..22: note = n is a, c, g, or t
  source 1..40: mol_type = other DNA
ctgtttggccgcggataggmnncacttcttgatcttccac

SEQ ID NO: 8 - DNA, 39 bp, synthetic construct
  misc_feature 19..20: note = n is a, c, g, or t
  source 1..39: mol_type = other DNA
ccgggtggtgaagtgatcnnkggtggtacctatttagtg

SEQ ID NO: 9 - DNA, 39 bp, synthetic construct
  misc_feature 20..21: note = n is a, c, g, or t
  source 1..39: mol_type = other DNA
cactaaataggtaccaccmnngatcacttcaccacccgg

SEQ ID NO: 10 - DNA, 40 bp, synthetic construct
  misc_feature 19..20: note = n is a, c, g, or t
  source 1..40: mol_type = other DNA
ggtaaagcaagccgtaccnnkccggttgttcatgcctatg

SEQ ID NO: 11 - DNA, 40 bp, synthetic construct
  misc_feature 21..22: note = n is a, c, g, or t
  source 1..40: mol_type = other DNA
cataggcatgaacaaccggmnnggtacggcttgctttacc

SEQ ID NO: 12 - DNA, 1116 bp, synthetic construct
  source 1..1116: mol_type = other DNA
atgacccagaataagcgcgtggttgttctgggcagtggcgttattggtctgagctgtgctttagctttagcccagaagggctataaagtgcatgtggttgcccgcgatctgccggaagacacagtggcccagacctttgcaagcccttgggccggtgcagcgtggaatccgcatatgagcaaagaagctggtccgcgtcaagctaaatgggaggaagcaaccttcaaacagtgggtggacttcgttccgcaaggtctggcaatgtggctgaaaggtacccgccgctttgcagaaaccgaagccgatctgctgggccattggtataaggacatcgtgccgaattaccgccatctgaacccgagcgattgtccgccgggcgcaattggcgtgacctacgatactttaagcgttaacgccccgaagttctgtcagtatctgcagcgcgaagcacagaaactgggcgtgaccttcgaacgccgtttagttacctctttagagcagattgcagatggcgccgatctgatcgttaatgcaaccggtctgggcgccaaaagcatcgccggtgtggaagatcaagaagtggaacctatccgcggccaaacagtgctgattaagagcaactgtaaacgcctgaccactgacagtagtgacccgaaaagcccggcctacattattccgcgcccgggtggtgaagtgatctgtggtggtacctatttagtgggtaactatgatttaagcgtggatccggccaccattccgcgcattttaaaacattgtctgcgtttagacccgagtattagcaccgacggcacactggaaggcatcgaaattttacgccataacgttggtctgcgtcccgctcgtcgtggtggtccgcgtgtggaattagaacgcgtgagcttcccgctgaagcgcggtcagagtctgttagctttaggcaccgccaaagcagcagaaggtaaagcaagccgtaccgtgccggttgttcatgcctatggcttcagcagcgccggttaccaacaaggttggggcgcagctttagaagttcgtgatctggtggaccaagctattggtagcagcagtagtgccagtagtggccgttatttagccaaactg